European Patent Application EP 4 810 613 A1, published September 23, 2026. Title: 一种抵抗带状疱疹的mRNA 疫苗及其制备方法. Applicant: 石药集团巨石生物制药有限公司. Application CN. The sequence listing filed with the application follows.

SEQUENCE LISTING (18 sequences)

SEQ ID NO: 1 - RNA, 2224 nt, synthetic construct
  source 1..2224: mol_type = other RNA
gggagacccaagctggctagcgtttaaacttaagcttggtaccgagctcggatccactagtccagtgtggtggaattcgggaaataagagagaaaagaagagtaagaagaaatataagagccaccatggggacagttaataaacctgtggtgggggtattgatggggttcggaattatcacgggaacgttgcgtataacgaatccggtcagagcatccgtcttgcgatacgatgattttcacaccgatgaagacaaactggatacaaactccgtatatgagccttactaccattcagatcatgcggagtcttcatgggtaaatcggggagagtcttcgcgaaaagcgtacgatcataactcaccttatatatggccacgtaatgattatgatggatttttagagaacgcacacgaacaccatggggtgtataatcagggccgtggtatcgatagcggggaacggttaatgcaacccacacaaatgtctgcacaggaggatcttggggacgatacgggcatccacgttatccctacgttaaacggcgatgacagacataaaattgtaaatgtggaccaacgtcaatacggtgacgtgtttaaaggagatcttaatccaaaaccccaaggccaaagactcattgaggtgtcagtggaagaaaatcacccgtttactttacgcgcaccgattcagcggatttatggagtccggtacaccgagacttggagctttttgccgtcattaacctgtacgggagacgcagcgcccgccatccagcatatatgtttaaaacatacaacatgctttcaagacgtggtggtggatgtggattgcgcggaaaatactaaagaggatcagttggccgaaatcagttaccgttttcaaggtaagaaggaagcggaccaaccgtggattgttgtaaacacgagcacactgtttgatgaactcgaattagacccccccgagattgaaccgggtgtcttgaaagtacttcggacagaaaaacaatacttgggtgtgtacatttggaacatgcgcggctccgatggtacgtctacctacgccacgtttttggtcacctggaaaggggatgaaaaaacaagaaaccctacgcccgcagtaactcctcaaccaagaggggctgagtttcatatgtggaattaccactcgcatgtattttcagttggtgatacgtttagcttggcaatgcatcttcagtataagatacatgaagcgccatttgatttgctgttagagtggttgtatgtccccatcgatcctacatgtcaaccaatgcggttatattctacgtgtttgtatcatcccaacgcaccccaatgcctctctcatatgaattccggttgtacatttacctcgccacatttagcccagcgtgttgcaagcacagtgtatcaaaattgtgaacatgcagataactacaccgcatattgtctgggaatatctcatatggagcctagctttggtctaatcttacacgacgggggcaccacgttaaagtttgtagatacacccgagagtttgtcgggattatacgtttttgtggtgtattttaacgggcatgttgaagccgtagcatacactgttgtatccacagtagatcattttgtaaacgcaattgaagagcgtggatttccgccaacggccggtcagccaccggcgactactaaacccaaggaaattacccccgtaaaccccggaacgtcaccacttctacgatatgccgcatggaccggagggcttgcagcagtagtacttttatgtctcgtaatatttttaatctgtacggctaaacgaatgagggttaaagcctatagggtagacaagtccccgtataaccaaagcatgtattacgctggccttccagtggacgatttcgaggactcggaatctacggatacggaagaagagtttggtaacgcgattggagggagtcacgggggttcgagttacacggtgtatatagataagacccggtgataataggctggagcctcggtggccatgcttcttgccccttgggcctccccccagcccctcctccccttcctgcacccgtacccccgtggtctttgaataaagtctgagtgggcggcaaaaaaaaaaaaaaaaaaaaaaaaaaaaaaagcatatgactaaaaaaaaaaaaaaaaaaaaaaaaaaaaaaaaaaaaaaaaaaaaaaaaaaaaaaaaaaaaaaaaaaaaaa

SEQ ID NO: 2 - RNA, 2224 nt, synthetic construct
  source 1..2224: mol_type = other RNA
gggagacccaagctggctagcgtttaaacttaagcttggtaccgagctcggatccactagtccagtgtggtggaattcgggaaataagagagaaaagaagagtaagaagaaatataagagccaccatgggcaccgtgaacaagcccgtggtgggcgtgctgatgggcttcggcatcatcaccggcaccctgcggatcaccaaccccgtgcgggccagcgtgctgcggtacgacgacttccacaccgacgaggacaagctggacaccaacagcgtgtacgagccctactaccacagcgaccacgccgagagcagctgggtgaaccggggcgagagctcccggaaggcctacgaccacaacagcccctacatctggccccggaacgactacgacggcttcctggagaacgcccacgagcaccacggcgtgtacaaccagggccggggcatcgacagcggcgagcggctgatgcagcccacccagatgagcgcccaggaggacctgggcgacgacaccggcatccacgtgatccccaccctgaacggcgacgaccggcacaagatcgtgaacgtggaccagcggcagtacggcgacgtgttcaagggcgacctgaaccccaagccccagggccagcggctgatcgaggtgagcgtggaggagaaccaccccttcaccctgcgggcccccatccagcggatctacggcgtgcggtacaccgagacctggagcttcctgcccagcctgacctgcaccggcgacgccgcccccgccatccagcacatctgcctgaagcacaccacctgcttccaggacgtggtggtggacgtggactgcgccgagaacaccaaggaggaccagctggccgagatcagctaccggttccagggcaagaaggaggccgaccagccctggatcgtggtgaacaccagcaccctgttcgacgagctggagctggacccccccgagatcgagcccggcgtgctgaaggtgctgcggaccgagaagcagtacctgggcgtgtacatctggaacatgcggggcagcgacggcaccagcacctacgccaccttcctggtgacctggaagggcgacgagaagacccgcaaccccacccccgccgtgaccccccagccccggggcgccgagttccacatgtggaactaccacagccacgtgttcagcgtgggcgacaccttcagcctggccatgcacctgcagtacaagatccacgaggcccccttcgacctgctgctggagtggctgtacgtgcccatcgaccccacctgccagcccatgcggctgtacagcacctgcctgtaccaccccaacgccccccagtgcctgagccacatgaacagcggctgcaccttcaccagcccccacctggcccagcgggtggccagcaccgtgtaccagaactgcgagcacgccgacaactacaccgcctactgcctgggcatcagccacatggagcccagcttcggcctgatcctgcacgacggcggcaccaccctgaagttcgtggacacccccgagagcctgagcggcctgtacgtgttcgtggtgtacttcaacggccacgtggaggccgtggcctacaccgtggtgagcaccgtggaccacttcgtgaacgccatcgaggagcggggcttcccccccaccgccggccagccccccgccaccaccaagcccaaggagatcacccccgtgaaccccggcaccagccccctgctgcggtacgccgcctggaccggcggcctggccgccgtggtgctgctgtgcctggtgatcttcctgatctgcaccgccaagcggatgcgggtgaaggcctaccgggtggacaagagcccctacaaccagagcatgtactacgccggcctgcccgtggacgacttcgaggacagcgagagcaccgacaccgaggaggagttcggcaacgccatcggcggcagccacggcggcagcagctacaccgtgtacatcgacaagacccgctgataataggctggagcctcggtggccatgcttcttgccccttgggcctccccccagcccctcctccccttcctgcacccgtacccccgtggtctttgaataaagtctgagtgggcggcaaaaaaaaaaaaaaaaaaaaaaaaaaaaaaagcatatgactaaaaaaaaaaaaaaaaaaaaaaaaaaaaaaaaaaaaaaaaaaaaaaaaaaaaaaaaaaaaaaaaaaaaaa

SEQ ID NO: 3 - RNA, 2032 nt, synthetic construct
  source 1..2032: mol_type = other RNA
gggagacccaagctggctagcgtttaaacttaagcttggtaccgagctcggatccactagtccagtgtggtggaattcgggaaataagagagaaaagaagagtaagaagaaatataagagccaccatgggcacagtaaataaaccagttgttggagtgctgatggggttcggcatcatcaccggcaccctgcggatcaccaaccccgtgcgggccagcgtgctgcggtacgacgacttccacaccgacgaggacaagctggacaccaacagcgtgtacgagccctactaccacagcgaccacgccgagagcagctgggtgaaccggggcgagagcagccggaaggcctacgaccacaacagcccctacatctggccccggaacgactacgacggcttcctggagaacgcccacgagcaccacggcgtgtacaaccagggccggggcatcgactccggcgagcggctgatgcagcccacccagatgagcgcccaggaggacctgggcgacgacaccggcatccacgtgatccccaccctgaacggcgacgaccggcacaagatcgtgaacgtggaccagcggcagtacggcgacgtgttcaagggcgacctgaaccccaagccccagggccagcggctgatcgaggtgagcgtggaggagaaccaccccttcaccctgcgggcccccatccagcggatctacggcgtgcggtacaccgagacctggagcttcctgcccagcctgacctgcaccggcgacgccgcccccgccatccagcacatctgcctgaagcacaccacctgcttccaggacgtggtggtggacgtggactgcgccgagaacaccaaggaggaccagctggccgagatcagctaccggttccagggcaagaaggaggccgaccagccctggatcgtggtgaacaccagcaccctgttcgacgagctggagctggacccccccgagatcgagcccggcgtgctgaaggtgctgcggaccgagaagcagtacctgggcgtgtacatctggaacatgcggggcagcgacggcaccagcacctacgccaccttcctggtgacctggaagggcgacgagaagacccggaaccccacccccgccgtgaccccccagccccggggcgccgagttccacatgtggaactaccacagccacgtgttcagcgtgggcgacaccttcagcctggccatgcacctgcagtacaagatccacgaggcccccttcgacctgctgctggagtggctgtacgtgcccatcgaccccacctgccagcccatgcggctgtacagcacctgcctgtaccaccccaacgccccccagtgcctgagccacatgaacagcggctgcaccttcacctccccccacctggcccagcgggtggccagcaccgtgtaccagaactgcgagcacgccgacaactacaccgcctactgcctgggcatcagccacatggagcccagcttcggcctgatcctgcacgacggcggcaccaccctgaagttcgtggacacccccgagagcctgagcggcctgtacgtgttcgtggtgtacttcaacggccacgtggaggccgtggcctacaccgtggtgagcaccgtggaccacttcgtgaacgccatcgaggagcggggcttcccccccaccgccggccagccccccgccaccaccaagcccaaggagatcacccccgtgaaccccggcaccagccccctgctgcggtacgccgcctggaccggcggcctggccgccgtggtgctgctgtgcctggtgatcttcctgatctgctgataataggctggagcctcggtggccatgcttcttgccccttgggcctccccccagcccctcctccccttcctgcacccgtacccccgtggtctttgaataaagtctgagtgggcggcaaaaaaaaaaaaaaaaaaaaaaaaaaaaaaagcatatgactaaaaaaaaaaaaaaaaaaaaaaaaaaaaaaaaaaaaaaaaaaaaaaaaaaaaaaaaaaaaaaaaaaaaaa

SEQ ID NO: 4 - RNA, 2224 nt, synthetic construct
  source 1..2224: mol_type = other RNA
gggagacccaagctggctagcgtttaaacttaagcttggtaccgagctcggatccactagtccagtgtggtggaattcgggaaataagagagaaaagaagagtaagaagaaatataagagccaccatgggaacagtaaataaaccagttgttggagtgctgatgggcttcggcatcatcaccggcaccctgcggatcaccaaccccgtgcgcgccagcgtgctgcggtacgacgacttccacaccgacgaggacaagctggacaccaacagcgtgtacgagccctactaccacagcgaccacgccgagagcagctgggtgaaccggggcgagagcagccggaaggcctacgaccacaacagcccctacatctggccccggaacgactacgacggcttcctggagaacgcccacgagcaccacggcgtgtacaaccagggccggggcatcgacagcggcgagcggctgatgcagcccacccagatgagcgcccaggaggacctgggcgacgacaccggcatccacgtgatccccaccctgaacggcgacgaccggcacaagatcgtgaacgtggaccagcggcagtacggcgacgtgttcaagggcgacctgaaccccaagccccagggccagcggctgatcgaggtgagcgtggaggagaaccaccccttcaccctgcgggcccccatccagcggatctacggcgtgcggtacaccgagacctggagcttcctgcccagcctgacctgcaccggcgacgccgcccccgccatccagcacatctgcctgaagcacaccacctgcttccaggacgtggtggtggacgtggactgcgccgagaacaccaaggaggaccagctggccgagatcagctaccggttccagggcaagaaggaggccgaccagccctggatcgtggtgaacaccagcaccctgttcgacgagctggagctggacccccccgagatcgagcccggcgtgctgaaggtgctgcggaccgagaagcagtacctgggcgtgtacatctggaacatgcggggcagcgacggcaccagcacctacgccaccttcctggtgacctggaagggcgacgagaagacccggaaccccacccccgccgtgaccccccagccccggggcgccgagttccacatgtggaactaccacagccacgtgttcagcgtgggcgacaccttcagcctggccatgcacctgcagtacaagatccacgaggcccccttcgacctgctgctggagtggctgtacgtgcccatcgaccccacctgccagcccatgcggctgtacagcacctgcctgtaccaccccaacgccccccagtgcctgagccacatgaacagcggctgcaccttcaccagcccccacctggcccagcgggtggccagcaccgtgtaccagaactgcgagcacgccgacaactacaccgcctactgcctgggcatcagccacatggagcccagcttcggcctgatcctgcacgacggcggcaccaccctgaagttcgtggacacccccgagagcctgagcggcctgtacgtgttcgtggtgtacttcaacggccacgtggaggccgtggcctacaccgtggtgagcaccgtggaccacttcgtgaacgccatcgaggagcggggcttcccccccaccgccggccagccccccgccaccaccaagcccaaggagatcacccccgtgaaccccggcaccagccccctgctgcggtacgccgcctggaccggcggcctggccgccgtggtgctgctgtgcctggtgatcttcctgatctgcaccgccaagcggatgcgggtgaaggcctaccgggtggacaagagcccctacaaccagagcatgtactacgccggcctgcccgtggacgacttcgaggacctggagctgctggacctggaggaggagttcggcaacgccatcggcggcagccacggcggcagcagctacaccgtgtacatcgacaagacccggtgataataggctggagcctcggtggccatgcttcttgccccttgggcctccccccagcccctcctccccttcctgcacccgtacccccgtggtctttgaataaagtctgagtgggcggcaaaaaaaaaaaaaaaaaaaaaaaaaaaaaaagcatatgactaaaaaaaaaaaaaaaaaaaaaaaaaaaaaaaaaaaaaaaaaaaaaaaaaaaaaaaaaaaaaaaaaaaaaa

SEQ ID NO: 5 - RNA, 2224 nt, synthetic construct
  source 1..2224: mol_type = other RNA
gggagacccaagctggctagcgtttaaacttaagcttggtaccgagctcggatccactagtccagtgtggtggaattcgggaaataagagagaaaagaagagtaagaagaaatataagagccaccatgggcacagttaataaaccagtagttggagtgctgatgggcttcgggatcatcaccggcaccctgcggatcaccaaccccgtgcgggccagcgtgctgcggtacgacgacttccacaccgacgaggacaagctggacaccaacagcgtgtacgagccctactaccacagcgaccacgccgagagcagctgggtgaaccggggcgagagcagccggaaggcctacgaccacaacagcccctacatctggccccggaacgactacgacggcttcctggagaacgcccacgagcaccacggcgtgtacaaccagggccggggcatcgactccggcgagcggctgatgcagcccacccagatgagcgcccaggaggacctgggcgacgacaccggcatccacgtgatccccaccctgaacggcgacgaccggcacaagatcgtgaacgtggaccagcggcagtacggcgacgtgttcaagggcgacctgaaccccaagccccagggccagcggctgatcgaggtgagcgtggaggagaaccaccccttcaccctgcgggcccccatccagcggatctacggcgtgcggtacaccgagacctggagcttcctgcccagcctgacctgcaccggcgacgccgcccccgccatccagcacatctgcctgaagcacaccacctgcttccaggacgtggtggtggacgtggactgcgccgagaacaccaaggaggaccagctggccgagatcagctaccggttccagggcaagaaggaggccgaccagccctggatcgtggtgaacaccagcaccctgttcgacgagctggagctggacccccccgagatcgagcccggcgtgctgaaggtgctgcggaccgagaagcagtacctgggcgtgtacatctggaacatgcggggcagcgacggcaccagcacctacgccaccttcctggtgacctggaagggcgacgagaagacccggaaccccacccccgccgtgaccccccagccccggggcgccgagttccacatgtggaactaccacagccacgtgttcagcgtgggcgacaccttcagcctggccatgcacctgcagtacaagatccacgaggcccccttcgacctgctgctggagtggctgtacgtgcccatcgaccccacctgccagcccatgcggctgtacagcacctgcctgtaccaccccaacgccccccagtgcctgagccacatgaacagcggctgcaccttcaccagcccccacctggcccagcgggtggccagcaccgtgtaccagaactgcgagcacgccgacaactacaccgcctactgcctgggcatcagccacatggagcccagcttcggcctgatcctgcacgacggcggcaccaccctgaagttcgtggacacccccgagagcctgagcggcctgtacgtgttcgtggtgtacttcaacggccacgtggaggccgtggcctacaccgtggtgagcaccgtggaccacttcgtgaacgccatcgaggagcggggcttcccccccaccgccggccagccccccgccaccaccaagcccaaggagatcacccccgtgaaccccggcaccagccccctgctgcggtacgccgcctggaccggcggcctggccgccgtggtgctgctgtgcctggtgatcttcctgatctgcaccgccaagcggatgcgggtgaaggcctaccgggtggacaagagcccctacaaccagagcatgtactacgccggcctgcccgtggacgacttcgaggacatcgagatcatcgacatcgaggaggagttcggcaacgccatcggcggcagccacggcggctccagctacaccgtgtacatcgacaagacccggtgataataggctggagcctcggtggccatgcttcttgccccttgggcctccccccagcccctcctccccttcctgcacccgtacccccgtggtctttgaataaagtctgagtgggcggcaaaaaaaaaaaaaaaaaaaaaaaaaaaaaaagcatatgactaaaaaaaaaaaaaaaaaaaaaaaaaaaaaaaaaaaaaaaaaaaaaaaaaaaaaaaaaaaaaaaaaaaaaa

SEQ ID NO: 6 - RNA, 2224 nt, synthetic construct
  source 1..2224: mol_type = other RNA
gggagacccaagctggctagcgtttaaacttaagcttggtaccgagctcggatccactagtccagtgtggtggaattcgggaaataagagagaaaagaagagtaagaagaaatataagagccaccatgggaacagtaaataaaccagttgttggagtgctgatgggcttcggcatcatcaccggcaccctgcggatcaccaaccccgtgcgcgccagcgtgctgcggtacgacgacttccacaccgacgaggacaagctggacaccaacagcgtgtacgagccctactaccacagcgaccacgccgagagcagctgggtgaaccggggcgagagcagccggaaggcctacgaccacaacagcccctacatctggccccggaacgactacgacggcttcctggagaacgcccacgagcaccacggcgtgtacaaccagggccggggcatcgacagcggcgagcggctgatgcagcccacccagatgagcgcccaggaggacctgggcgacgacaccggcatccacgtgatccccaccctgaacggcgacgaccggcacaagatcgtgaacgtggaccagcggcagtacggcgacgtgttcaagggcgacctgaaccccaagccccagggccagcggctgatcgaggtgagcgtggaggagaaccaccccttcaccctgcgggcccccatccagcggatctacggcgtgcggtacaccgagacctggagcttcctgcccagcctgacctgcaccggcgacgccgcccccgccatccagcacatctgcctgaagcacaccacctgcttccaggacgtggtggtggacgtggactgcgccgagaacaccaaggaggaccagctggccgagatcagctaccggttccagggcaagaaggaggccgaccagccctggatcgtggtgaacaccagcaccctgttcgacgagctggagctggacccccccgagatcgagcccggcgtgctgaaggtgctgcggaccgagaagcagtacctgggcgtgtacatctggaacatgcggggcagcgacggcaccagcacctacgccaccttcctggtgacctggaagggcgacgagaagacccggaaccccacccccgccgtgaccccccagccccggggcgccgagttccacatgtggaactaccacagccacgtgttcagcgtgggcgacaccttcagcctggccatggagctgcagtacaagatccacgaggcccccttcgacctgctgctggagtggctgtacgtgcccatcgaccccacctgccagcccatgcggctgtacagcacctgcctgtaccaccccaacgccccccagtgcctgagccacatgaacagcggctgcaccttcaccagcccccacctggcccagcgggtggccagcaccgtgtaccagaactgcgagcacgccgacaactacaccgcctactgcctgggcatcagccacatggagcccagcttcggcctgatcctgcacgacggcggcaccaccctgaagttcgtggacacccccgagagcctgagcggcctgtacgtgttcgtggtgtacttcaacggccacgtggaggccgtggcctacaccgtggtgagcaccgtggaccacttcgtgaacgccatcgaggagcggggcttcccccccaccgccggccagccccccgccaccaccaagcccaaggagatcacccccgtgaaccccggcaccagccccctgctgcggtacgccgcctggaccggcggcctggccgccgtggtgctgctgtgcctggtgatcttcctgatctgcaccgccaagcggatgcgggtgaaggcctaccgggtggacaagagcccctacaaccagagcatgtactacgccggcctgcccgtggacgacttcgaggacctggagctgctggacctggaggaggagttcggcaacgccatcggcggcagccacggcggcagcagctacaccgtgtacatcgacaagacccggtgataataggctggagcctcggtggccatgcttcttgccccttgggcctccccccagcccctcctccccttcctgcacccgtacccccgtggtctttgaataaagtctgagtgggcggcaaaaaaaaaaaaaaaaaaaaaaaaaaaaaaagcatatgactaaaaaaaaaaaaaaaaaaaaaaaaaaaaaaaaaaaaaaaaaaaaaaaaaaaaaaaaaaaaaaaaaaaaaa

SEQ ID NO: 7 - RNA, 2224 nt, synthetic construct
  source 1..2224: mol_type = other RNA
gggagacccaagctggctagcgtttaaacttaagcttggtaccgagctcggatccactagtccagtgtggtggaattcgggaaataagagagaaaagaagagtaagaagaaatataagagccaccatgggcacagttaataaaccagtagttggagtgctgatgggcttcgggatcatcaccggcaccctgcggatcaccaaccccgtgcgggccagcgtgctgcggtacgacgacttccacaccgacgaggacaagctggacaccaacagcgtgtacgagccctactaccacagcgaccacgccgagagcagctgggtgaaccggggcgagagcagccggaaggcctacgaccacaacagcccctacatctggccccggaacgactacgacggcttcctggagaacgcccacgagcaccacggcgtgtacaaccagggccggggcatcgactccggcgagcggctgatgcagcccacccagatgagcgcccaggaggacctgggcgacgacaccggcatccacgtgatccccaccctgaacggcgacgaccggcacaagatcgtgaacgtggaccagcggcagtacggcgacgtgttcaagggcgacctgaaccccaagccccagggccagcggctgatcgaggtgagcgtggaggagaaccaccccttcaccctgcgggcccccatccagcggatctacggcgtgcggtacaccgagacctggagcttcctgcccagcctgacctgcaccggcgacgccgcccccgccatccagcacatctgcctgaagcacaccacctgcttccaggacgtggtggtggacgtggactgcgccgagaacaccaaggaggaccagctggccgagatcagctaccggttccagggcaagaaggaggccgaccagccctggatcgtggtgaacaccagcaccctgttcgacgagctggagctggacccccccgagatcgagcccggcgtgctgaaggtgctgcggaccgagaagcagtacctgggcgtgtacatctggaacatgcggggcagcgacggcaccagcacctacgccaccttcctggtgacctggaagggcgacgagaagacccggaaccccacccccgccgtgaccccccagccccggggcgccgagttccacatgtggaactaccacagccacgtgttcagcgtgggcgacaccttcagcctggccatggagctgcagtacaagatccacgaggcccccttcgacctgctgctggagtggctgtacgtgcccatcgaccccacctgccagcccatgcggctgtacagcacctgcctgtaccaccccaacgccccccagtgcctgagccacatgaacagcggctgcaccttcaccagcccccacctggcccagcgggtggccagcaccgtgtaccagaactgcgagcacgccgacaactacaccgcctactgcctgggcatcagccacatggagcccagcttcggcctgatcctgcacgacggcggcaccaccctgaagttcgtggacacccccgagagcctgagcggcctgtacgtgttcgtggtgtacttcaacggccacgtggaggccgtggcctacaccgtggtgagcaccgtggaccacttcgtgaacgccatcgaggagcggggcttcccccccaccgccggccagccccccgccaccaccaagcccaaggagatcacccccgtgaaccccggcaccagccccctgctgcggtacgccgcctggaccggcggcctggccgccgtggtgctgctgtgcctggtgatcttcctgatctgcaccgccaagcggatgcgggtgaaggcctaccgggtggacaagagcccctacaaccagagcatgtactacgccggcctgcccgtggacgacttcgaggacatcgagatcatcgacatcgaggaggagttcggcaacgccatcggcggcagccacggcggctccagctacaccgtgtacatcgacaagacccggtgataataggctggagcctcggtggccatgcttcttgccccttgggcctccccccagcccctcctccccttcctgcacccgtacccccgtggtctttgaataaagtctgagtgggcggcaaaaaaaaaaaaaaaaaaaaaaaaaaaaaaagcatatgactaaaaaaaaaaaaaaaaaaaaaaaaaaaaaaaaaaaaaaaaaaaaaaaaaaaaaaaaaaaaaaaaaaaaaa

SEQ ID NO: 8 - protein, 623 aa, synthetic construct
MGTVNKPVVGVLMGFGIITGTLRITNPVRASVLRYDDFHTDEDKLDTNSVYEPYYHSDHAESSWVNRGESSRKAYDHNSPYIWPRNDYDGFLENAHEHHGVYNQGRGIDSGERLMQPTQMSAQEDLGDDTGIHVIPTLNGDDRHKIVNVDQRQYGDVFKGDLNPKPQGQRLIEVSVEENHPFTLRAPIQRIYGVRYTETWSFLPSLTCTGDAAPAIQHICLKHTTCFQDVVVDVDCAENTKEDQLAEISYRFQGKKEADQPWIVVNTSTLFDELELDPPEIEPGVLKVLRTEKQYLGVYIWNMRGSDGTSTYATFLVTWKGDEKTRNPTPAVTPQPRGAEFHMWNYHSHVFSVGDTFSLAMHLQYKIHEAPFDLLLEWLYVPIDPTCQPMRLYSTCLYHPNAPQCLSHMNSGCTFTSPHLAQRVASTVYQNCEHADNYTAYCLGISHMEPSFGLILHDGGTTLKFVDTPESLSGLYVFVVYFNGHVEAVAYTVVSTVDHFVNAIEERGFPPTAGQPPATTKPKEITPVNPGTSPLLRYAAWTGGLAAVVLLCLVIFLICTAKRMRVKAYRVDKSPYNQSMYYAGLPVDDFEDSESTDTEEEFGNAIGGSHGGSSYTVYIDKTR

SEQ ID NO: 9 - skipped

SEQ ID NO: 10 - RNA, 125 nt, synthetic construct
  source 1..125: mol_type = other RNA
gggagacccaagctggctagcgtttaaacttaagcttggtaccgagctcggatccactagtccagtgtggtggaattcgggaaataagagagaaaagaagagtaagaagaaatataagagccacc

SEQ ID NO: 11 - RNA, 110 nt, synthetic construct
  source 1..110: mol_type = other RNA
aaaaaaaaaaaaaaaaaaaaaaaaaaaaaagcatatgactaaaaaaaaaaaaaaaaaaaaaaaaaaaaaaaaaaaaaaaaaaaaaaaaaaaaaaaaaaaaaaaaaaaaaa

SEQ ID NO: 12 - RNA, 110 nt, synthetic construct
  source 1..110: mol_type = other RNA
gctggagcctcggtggccatgcttcttgccccttgggcctccccccagcccctcctccccttcctgcacccgtacccccgtggtctttgaataaagtctgagtgggcggc

SEQ ID NO: 13 - protein, 559 aa, synthetic construct
MGTVNKPVVGVLMGFGIITGTLRITNPVRASVLRYDDFHTDEDKLDTNSVYEPYYHSDHAESSWVNRGESSRKAYDHNSPYIWPRNDYDGFLENAHEHHGVYNQGRGIDSGERLMQPTQMSAQEDLGDDTGIHVIPTLNGDDRHKIVNVDQRQYGDVFKGDLNPKPQGQRLIEVSVEENHPFTLRAPIQRIYGVRYTETWSFLPSLTCTGDAAPAIQHICLKHTTCFQDVVVDVDCAENTKEDQLAEISYRFQGKKEADQPWIVVNTSTLFDELELDPPEIEPGVLKVLRTEKQYLGVYIWNMRGSDGTSTYATFLVTWKGDEKTRNPTPAVTPQPRGAEFHMWNYHSHVFSVGDTFSLAMHLQYKIHEAPFDLLLEWLYVPIDPTCQPMRLYSTCLYHPNAPQCLSHMNSGCTFTSPHLAQRVASTVYQNCEHADNYTAYCLGISHMEPSFGLILHDGGTTLKFVDTPESLSGLYVFVVYFNGHVEAVAYTVVSTVDHFVNAIEERGFPPTAGQPPATTKPKEITPVNPGTSPLLRYAAWTGGLAAVVLLCLVIFLIC

SEQ ID NO: 14 - protein, 623 aa, synthetic construct
MGTVNKPVVGVLMGFGIITGTLRITNPVRASVLRYDDFHTDEDKLDTNSVYEPYYHSDHAESSWVNRGESSRKAYDHNSPYIWPRNDYDGFLENAHEHHGVYNQGRGIDSGERLMQPTQMSAQEDLGDDTGIHVIPTLNGDDRHKIVNVDQRQYGDVFKGDLNPKPQGQRLIEVSVEENHPFTLRAPIQRIYGVRYTETWSFLPSLTCTGDAAPAIQHICLKHTTCFQDVVVDVDCAENTKEDQLAEISYRFQGKKEADQPWIVVNTSTLFDELELDPPEIEPGVLKVLRTEKQYLGVYIWNMRGSDGTSTYATFLVTWKGDEKTRNPTPAVTPQPRGAEFHMWNYHSHVFSVGDTFSLAMHLQYKIHEAPFDLLLEWLYVPIDPTCQPMRLYSTCLYHPNAPQCLSHMNSGCTFTSPHLAQRVASTVYQNCEHADNYTAYCLGISHMEPSFGLILHDGGTTLKFVDTPESLSGLYVFVVYFNGHVEAVAYTVVSTVDHFVNAIEERGFPPTAGQPPATTKPKEITPVNPGTSPLLRYAAWTGGLAAVVLLCLVIFLICTAKRMRVKAYRVDKSPYNQSMYYAGLPVDDFEDIEIIDIEEEFGNAIGGSHGGSSYTVYIDKTR

SEQ ID NO: 15 - protein, 623 aa, synthetic construct
MGTVNKPVVGVLMGFGIITGTLRITNPVRASVLRYDDFHTDEDKLDTNSVYEPYYHSDHAESSWVNRGESSRKAYDHNSPYIWPRNDYDGFLENAHEHHGVYNQGRGIDSGERLMQPTQMSAQEDLGDDTGIHVIPTLNGDDRHKIVNVDQRQYGDVFKGDLNPKPQGQRLIEVSVEENHPFTLRAPIQRIYGVRYTETWSFLPSLTCTGDAAPAIQHICLKHTTCFQDVVVDVDCAENTKEDQLAEISYRFQGKKEADQPWIVVNTSTLFDELELDPPEIEPGVLKVLRTEKQYLGVYIWNMRGSDGTSTYATFLVTWKGDEKTRNPTPAVTPQPRGAEFHMWNYHSHVFSVGDTFSLAMELQYKIHEAPFDLLLEWLYVPIDPTCQPMRLYSTCLYHPNAPQCLSHMNSGCTFTSPHLAQRVASTVYQNCEHADNYTAYCLGISHMEPSFGLILHDGGTTLKFVDTPESLSGLYVFVVYFNGHVEAVAYTVVSTVDHFVNAIEERGFPPTAGQPPATTKPKEITPVNPGTSPLLRYAAWTGGLAAVVLLCLVIFLICTAKRMRVKAYRVDKSPYNQSMYYAGLPVDDFEDIEIIDIEEEFGNAIGGSHGGSSYTVYIDKTR

SEQ ID NO: 16 - protein, 623 aa, synthetic construct
MGTVNKPVVGVLMGFGIITGTLRITNPVRASVLRYDDFHTDEDKLDTNSVYEPYYHSDHAESSWVNRGESSRKAYDHNSPYIWPRNDYDGFLENAHEHHGVYNQGRGIDSGERLMQPTQMSAQEDLGDDTGIHVIPTLNGDDRHKIVNVDQRQYGDVFKGDLNPKPQGQRLIEVSVEENHPFTLRAPIQRIYGVRYTETWSFLPSLTCTGDAAPAIQHICLKHTTCFQDVVVDVDCAENTKEDQLAEISYRFQGKKEADQPWIVVNTSTLFDELELDPPEIEPGVLKVLRTEKQYLGVYIWNMRGSDGTSTYATFLVTWKGDEKTRNPTPAVTPQPRGAEFHMWNYHSHVFSVGDTFSLAMHLQYKIHEAPFDLLLEWLYVPIDPTCQPMRLYSTCLYHPNAPQCLSHMNSGCTFTSPHLAQRVASTVYQNCEHADNYTAYCLGISHMEPSFGLILHDGGTTLKFVDTPESLSGLYVFVVYFNGHVEAVAYTVVSTVDHFVNAIEERGFPPTAGQPPATTKPKEITPVNPGTSPLLRYAAWTGGLAAVVLLCLVIFLICTAKRMRVKAYRVDKSPYNQSMYYAGLPVDDFEDLELLDLEEEFGNAIGGSHGGSSYTVYIDKTR

SEQ ID NO: 17 - protein, 623 aa, synthetic construct
MGTVNKPVVGVLMGFGIITGTLRITNPVRASVLRYDDFHTDEDKLDTNSVYEPYYHSDHAESSWVNRGESSRKAYDHNSPYIWPRNDYDGFLENAHEHHGVYNQGRGIDSGERLMQPTQMSAQEDLGDDTGIHVIPTLNGDDRHKIVNVDQRQYGDVFKGDLNPKPQGQRLIEVSVEENHPFTLRAPIQRIYGVRYTETWSFLPSLTCTGDAAPAIQHICLKHTTCFQDVVVDVDCAENTKEDQLAEISYRFQGKKEADQPWIVVNTSTLFDELELDPPEIEPGVLKVLRTEKQYLGVYIWNMRGSDGTSTYATFLVTWKGDEKTRNPTPAVTPQPRGAEFHMWNYHSHVFSVGDTFSLAMELQYKIHEAPFDLLLEWLYVPIDPTCQPMRLYSTCLYHPNAPQCLSHMNSGCTFTSPHLAQRVASTVYQNCEHADNYTAYCLGISHMEPSFGLILHDGGTTLKFVDTPESLSGLYVFVVYFNGHVEAVAYTVVSTVDHFVNAIEERGFPPTAGQPPATTKPKEITPVNPGTSPLLRYAAWTGGLAAVVLLCLVIFLICTAKRMRVKAYRVDKSPYNQSMYYAGLPVDDFEDLELLDLEEEFGNAIGGSHGGSSYTVYIDKTR

SEQ ID NO: 18 - RNA, 47 nt, synthetic construct
  source 1..47: mol_type = other RNA
gggaaataagagagaaaagaagagtaagaagaaatataagagccacc